European Patent Application EP 4 474 394 A1, published December 11, 2024. Title: Neutralizing antibody against USAG-1 for tooth regeneration therapy. Applicant: Kyoto University UNIVERSITY OF FUKUI AICHI PREFECTURE OSAKA UNIVERSITY. The sequence listing filed with the application follows.

SEQUENCE LISTING (10 sequences)

SEQ ID NO: 1 - protein, 467 aa, Mus musculus
MKCSWVIFFLMAVVIGVNSEVQLQQSGAELVRPGASVKLSCTASGFNIKDDYMHWVKQRPEQGLEWIGWIDPENGDTEYASKFQGKATITADTSSNTAYLQLSSLTSEDTAVYYCITPYYYGSSFSYWYFDVWGTGTTVTVSSAKTTPPSVYPLAPGSAAQTNSMVTLGCLVKGYFPEPVTVTWNSGSLSSGVHTFPAVLQSDLYTLSSSVTVPSSTWPSQTVTCNVAHPASSTKVDKKIVPRDCGCKPCICTVPEVSSVFIFPPKPKDVLTITLTPKVTCVVVDISKDDPEVQFSWFVDDVEVHTAQTKPREEQINSTFRSVSELPIMHQDWLNGKEFKCRVNSAAFPAPIEKTISKTKGRPKAPQVYTIPPPKEQMAKDKVSLTCMITNFFPEDITVEWQWNGQPAENYKNTQPIMDTDGSYFVYSKLNVQKSNWEAGNTFTCSVLHEGLHNHHTEKSLSHSPGK

SEQ ID NO: 2 - protein, 238 aa, Mus musculus
MKLPVRLLVLMFWIPASSSDVLMTQTPLSLPVSLGDQASISCRSSQSIVHSNGNTYLEWYLQKPGQSPKLLIYKVSNRFSGVPDRFSGSGSGTDFTLKISRVEAEDLGVYYCFQGSHVPWTFGGGTKLEIKRADAAPTVSIFPPSSEQLTSGGASVVCFLNNFYPKDINVKWKIDGSERQNGVLNSWTDQDSKDSTYSMSSTLTLTKDEYERHNSYTCEATHKTSTSPIVKSFNRNEC

SEQ ID NO: 3 - protein, 124 aa, Mus musculus
EVQLQQSGAELVRPGASVKLSCTASGFNIKDDYMHWVKQRPEQGLEWIGWIDPENGDTEYASKFQGKATITADTSSNTAYLQLSSLTSEDTAVYYCITPYYYGSSFSYWYFDVWGTGTTVTVSS

SEQ ID NO: 4 - protein, 112 aa, Mus musculus
DVLMTQTPLSLPVSLGDQASISCRSSQSIVHSNGNTYLEWYLQKPGQSPKLLIYKVSNRFSGVPDRFSGSGSGTDFTLKISRVEAEDLGVYYCFQGSHVPWTFGGGTKLEIK

SEQ ID NO: 5 - protein, 8 aa, Mus musculus
GFNIKDDY

SEQ ID NO: 6 - protein, 8 aa, Mus musculus
IDPENGDT

SEQ ID NO: 7 - protein, 17 aa, Mus musculus
ITPYYYGSSFSYWYFDV

SEQ ID NO: 8 - protein, 16 aa, Mus musculus
RSSQSIVHSNGNTYLE

SEQ ID NO: 9 - protein, 7 aa, Mus musculus
KVSNRFS

SEQ ID NO: 10 - protein, 9 aa, Mus musculus
FQGSHVPWT